European Patent Specification EP 3 356 420 B1, published November 1, 2023. Title: MULTISPECIFIC ANTIBODIES. Applicant: F. Hoffmann-La Roche AG. The sequence listing filed with the application follows.

SEQUENCE LISTING (39 sequences)

SEQ ID NO: 1 - protein, 215 aa, Artificial
  7571 - kappa light chain (LC) <Ang-2> wild type (wt)
QPGLTQPPSVSVAPGQTARITCGGNNIGSKSVHWYQQKPGQAPVLVVYDDSDRPSGIPERFSGSNSGNTATLTISRVEAGDEADYYCQVWDSSSDHYVFGTGTKVTVLRTVAAPSVFIFPPSDEQLKSGTASVVCLLNNFYPREAKVQWKVDNALQSGNSQESVTEQDSKDSTYSLSSTLTLSKADYEKHKVYACEVTHQGLSSPVTKSFNRGEC

SEQ ID NO: 2 - protein, 459 aa, Artificial
  7595 - heavy chain (HC) <Ang-2> wild type (wt)
QVQLVESGAEVKKPGASVKVSCKASGYTFTGYYMHWVRQAPGQGLEWMGWINPNSGGTNYAQKFQGRVTMTRDTSISTAYMELSRLRSDDTAVYYCARSPNPYYYDSSGYYYPGAFDIWGQGTMVTVSSASTKGPSVFPLAPSSKSTSGGTAALGCLVKDYFPEPVTVSWNSGALTSGVHTFPAVLQSSGLYSLSSVVTVPSSSLGTQTYICNVNHKPSNTKVDKKVEPKSCDKTHTCPPCPAPELLGGPSVFLFPPKPKDTLMISRTPEVTCVVVDVSHEDPEVKFNWYVDGVEVHNAKTKPREEQYNSTYRVVSVLTVLHQDWLNGKEYKCKVSNKALPAPIEKTISKAKGQPREPQVYTLPPCRDELTKNQVSLWCLVKGFYPSDIAVEWESNGQPENNYKTTPPVLDSDGSFFLYSKLTVDKSRWQQGNVFSCSVMHEALHNHYTQKSLSLSPGK

SEQ ID NO: 3 - protein, 212 aa, Artificial
  7594 - light chain (LC) <VEGF> with CL-CH1 domain exchange wild type (wt)
DIQMTQSPSSLSASVGDRVTITCSASQDISNYLNWYQQKPGKAPKVLIYFTSSLHSGVPSRFSGSGSGTDFTLTISSLQPEDFATYYCQQYSTVPWTFGQGTKVEIKSSASTKGPSVFPLAPSSKSTSGGTAALGCLVKDYFPEPVTVSWNSGALTSGVHTFPAVLQSSGLYSLSSVVTVPSSSLGTQTYICNVNHKPSNTKVDKKVEPKSC

SEQ ID NO: 4 - protein, 457 aa, Artificial
  7593 - heavy chain (HC) <VEGF> with CL-CH1 domain exchange wild type (wt)
EVQLVESGGGLVQPGGSLRLSCAASGYTFTNYGMNWVRQAPGKGLEWVGWINTYTGEPTYAADFKRRFTFSLDTSKSTAYLQMNSLRAEDTAVYYCAKYPHYYGSSHWYFDVWGQGTLVTVSSASVAAPSVFIFPPSDEQLKSGTASVVCLLNNFYPREAKVQWKVDNALQSGNSQESVTEQDSKDSTYSLSSTLTLSKADYEKHKVYACEVTHQGLSSPVTKSFNRGECDKTHTCPPCPAPELLGGPSVFLFPPKPKDTLMISRTPEVTCVVVDVSHEDPEVKFNWYVDGVEVHNAKTKPREEQYNSTYRVVSVLTVLHQDWLNGKEYKCKVSNKALPAPIEKTISKAKGQPREPQVCTLPPSRDELTKNQVSLSCAVKGFYPSDIAVEWESNGQPENNYKTTPPVLDSDGSFFLVSKLTVDKSRWQQGNVFSCSVMHEALHNHYTQKSLSLSPGK

SEQ ID NO: 5 - protein, 215 aa, Artificial
  17914 - kappa light chain (LC) <Ang-2> with Q124K substitution
QPGLTQPPSVSVAPGQTARITCGGNNIGSKSVHWYQQKPGQAPVLVVYDDSDRPSGIPERFSGSNSGNTATLTISRVEAGDEADYYCQVWDSSSDHYVFGTGTKVTVLRTVAAPSVFIFPPSDEKLKSGTASVVCLLNNFYPREAKVQWKVDNALQSGNSQESVTEQDSKDSTYSLSSTLTLSKADYEKHKVYACEVTHQGLSSPVTKSFNRGEC

SEQ ID NO: 6 - protein, 459 aa, Artificial
  17911 - heavy chain (HC) <Ang-2> with K147E substitution
QVQLVESGAEVKKPGASVKVSCKASGYTFTGYYMHWVRQAPGQGLEWMGWINPNSGGTNYAQKFQGRVTMTRDTSISTAYMELSRLRSDDTAVYYCARSPNPYYYDSSGYYYPGAFDIWGQGTMVTVSSASTKGPSVFPLAPSSKSTSGGTAALGCLVEDYFPEPVTVSWNSGALTSGVHTFPAVLQSSGLYSLSSVVTVPSSSLGTQTYICNVNHKPSNTKVDKKVEPKSCDKTHTCPPCPAPELLGGPSVFLFPPKPKDTLMISRTPEVTCVVVDVSHEDPEVKFNWYVDGVEVHNAKTKPREEQYNSTYRVVSVLTVLHQDWLNGKEYKCKVSNKALPAPIEKTISKAKGQPREPQVYTLPPCRDELTKNQVSLWCLVKGFYPSDIAVEWESNGQPENNYKTTPPVLDSDGSFFLYSKLTVDKSRWQQGNVFSCSVMHEALHNHYTQKSLSLSPGK

SEQ ID NO: 7 - protein, 459 aa, Artificial
  17912 - heavy chain (HC) <Ang-2> with K213E substitution
QVQLVESGAEVKKPGASVKVSCKASGYTFTGYYMHWVRQAPGQGLEWMGWINPNSGGTNYAQKFQGRVTMTRDTSISTAYMELSRLRSDDTAVYYCARSPNPYYYDSSGYYYPGAFDIWGQGTMVTVSSASTKGPSVFPLAPSSKSTSGGTAALGCLVKDYFPEPVTVSWNSGALTSGVHTFPAVLQSSGLYSLSSVVTVPSSSLGTQTYICNVNHKPSNTKVDEKVEPKSCDKTHTCPPCPAPELLGGPSVFLFPPKPKDTLMISRTPEVTCVVVDVSHEDPEVKFNWYVDGVEVHNAKTKPREEQYNSTYRVVSVLTVLHQDWLNGKEYKCKVSNKALPAPIEKTISKAKGQPREPQVYTLPPCRDELTKNQVSLWCLVKGFYPSDIAVEWESNGQPENNYKTTPPVLDSDGSFFLYSKLTVDKSRWQQGNVFSCSVMHEALHNHYTQKSLSLSPGK

SEQ ID NO: 8 - protein, 215 aa, Artificial
  17913 - kappa light chain (LC) <Ang-2> with E123K substitution
QPGLTQPPSVSVAPGQTARITCGGNNIGSKSVHWYQQKPGQAPVLVVYDDSDRPSGIPERFSGSNSGNTATLTISRVEAGDEADYYCQVWDSSSDHYVFGTGTKVTVLRTVAAPSVFIFPPSDKQLKSGTASVVCLLNNFYPREAKVQWKVDNALQSGNSQESVTEQDSKDSTYSLSSTLTLSKADYEKHKVYACEVTHQGLSSPVTKSFNRGEC

SEQ ID NO: 9 - protein, 212 aa, Artificial
  17932 - light chain (LC) <VEGF> with CL-CH1 domain exchange and K147E substitution
DIQMTQSPSSLSASVGDRVTITCSASQDISNYLNWYQQKPGKAPKVLIYFTSSLHSGVPSRFSGSGSGTDFTLTISSLQPEDFATYYCQQYSTVPWTFGQGTKVEIKSSASTKGPSVFPLAPSSKSTSGGTAALGCLVEDYFPEPVTVSWNSGALTSGVHTFPAVLQSSGLYSLSSVVTVPSSSLGTQTYICNVNHKPSNTKVDKKVEPKSC

SEQ ID NO: 10 - protein, 457 aa, Artificial
  17934 - heavy chain (HC) <VEGF> with CL-CH1 domain exchange and Q124K substitution
EVQLVESGGGLVQPGGSLRLSCAASGYTFTNYGMNWVRQAPGKGLEWVGWINTYTGEPTYAADFKRRFTFSLDTSKSTAYLQMNSLRAEDTAVYYCAKYPHYYGSSHWYFDVWGQGTLVTVSSASVAAPSVFIFPPSDEKLKSGTASVVCLLNNFYPREAKVQWKVDNALQSGNSQESVTEQDSKDSTYSLSSTLTLSKADYEKHKVYACEVTHQGLSSPVTKSFNRGECDKTHTCPPCPAPELLGGPSVFLFPPKPKDTLMISRTPEVTCVVVDVSHEDPEVKFNWYVDGVEVHNAKTKPREEQYNSTYRVVSVLTVLHQDWLNGKEYKCKVSNKALPAPIEKTISKAKGQPREPQVCTLPPSRDELTKNQVSLSCAVKGFYPSDIAVEWESNGQPENNYKTTPPVLDSDGSFFLVSKLTVDKSRWQQGNVFSCSVMHEALHNHYTQKSLSLSPGK

SEQ ID NO: 11 - protein, 212 aa, Artificial
  17933 - light chain (LC) <VEGF> with CL-CH1 domain exchange and K213E substitution
DIQMTQSPSSLSASVGDRVTITCSASQDISNYLNWYQQKPGKAPKVLIYFTSSLHSGVPSRFSGSGSGTDFTLTISSLQPEDFATYYCQQYSTVPWTFGQGTKVEIKSSASTKGPSVFPLAPSSKSTSGGTAALGCLVKDYFPEPVTVSWNSGALTSGVHTFPAVLQSSGLYSLSSVVTVPSSSLGTQTYICNVNHKPSNTKVDEKVEPKSC

SEQ ID NO: 12 - protein, 215 aa, Artificial
  17301 - kappa light chain (LC) <Ang-2> with E123R and Q124K substitutions
QPGLTQPPSVSVAPGQTARITCGGNNIGSKSVHWYQQKPGQAPVLVVYDDSDRPSGIPERFSGSNSGNTATLTISRVEAGDEADYYCQVWDSSSDHYVFGTGTKVTVLRTVAAPSVFIFPPSDKRLKSGTASVVCLLNNFYPREAKVQWKVDNALQSGNSQESVTEQDSKDSTYSLSSTLTLSKADYEKHKVYACEVTHQGLSSPVTKSFNRGEC

SEQ ID NO: 13 - protein, 459 aa, Artificial
  14116 - heavy chain (HC) <Ang-2> with K147E and K213E substitutions
QVQLVESGAEVKKPGASVKVSCKASGYTFTGYYMHWVRQAPGQGLEWMGWINPNSGGTNYAQKFQGRVTMTRDTSISTAYMELSRLRSDDTAVYYCARSPNPYYYDSSGYYYPGAFDIWGQGTMVTVSSASTKGPSVFPLAPSSKSTSGGTAALGCLVEDYFPEPVTVSWNSGALTSGVHTFPAVLQSSGLYSLSSVVTVPSSSLGTQTYICNVNHKPSNTKVDEKVEPKSCDKTHTCPPCPAPELLGGPSVFLFPPKPKDTLMISRTPEVTCVVVDVSHEDPEVKFNWYVDGVEVHNAKTKPREEQYNSTYRVVSVLTVLHQDWLNGKEYKCKVSNKALPAPIEKTISKAKGQPREPQVYTLPPCRDELTKNQVSLWCLVKGFYPSDIAVEWESNGQPENNYKTTPPVLDSDGSFFLYSKLTVDKSRWQQGNVFSCSVMHEALHNHYTQKSLSLSPGK

SEQ ID NO: 14 - protein, 459 aa, Artificial
  17305 - heavy chain (HC) <Ang-2> with K147E and K213D substitutions
QVQLVESGAEVKKPGASVKVSCKASGYTFTGYYMHWVRQAPGQGLEWMGWINPNSGGTNYAQKFQGRVTMTRDTSISTAYMELSRLRSDDTAVYYCARSPNPYYYDSSGYYYPGAFDIWGQGTMVTVSSASTKGPSVFPLAPSSKSTSGGTAALGCLVEDYFPEPVTVSWNSGALTSGVHTFPAVLQSSGLYSLSSVVTVPSSSLGTQTYICNVNHKPSNTKVDDKVEPKSCDKTHTCPPCPAPELLGGPSVFLFPPKPKDTLMISRTPEVTCVVVDVSHEDPEVKFNWYVDGVEVHNAKTKPREEQYNSTYRVVSVLTVLHQDWLNGKEYKCKVSNKALPAPIEKTISKAKGQPREPQVYTLPPCRDELTKNQVSLWCLVKGFYPSDIAVEWESNGQPENNYKTTPPVLDSDGSFFLYSKLTVDKSRWQQGNVFSCSVMHEALHNHYTQKSLSLSPGK

SEQ ID NO: 15 - protein, 215 aa, Artificial
  17953 - kappa light chain (LC) <Ang-2> with Q38E, E123K and Q124K substitutions
QPGLTQPPSVSVAPGQTARITCGGNNIGSKSVHWYQEKPGQAPVLVVYDDSDRPSGIPERFSGSNSGNTATLTISRVEAGDEADYYCQVWDSSSDHYVFGTGTKVTVLRTVAAPSVFIFPPSDKKLKSGTASVVCLLNNFYPREAKVQWKVDNALQSGNSQESVTEQDSKDSTYSLSSTLTLSKADYEKHKVYACEVTHQGLSSPVTKSFNRGEC

SEQ ID NO: 16 - protein, 459 aa, Artificial
  17954 - heavy chain (HC) <Ang-2> with Q39K, K147E and K213E substitutions
QVQLVESGAEVKKPGASVKVSCKASGYTFTGYYMHWVRKAPGQGLEWMGWINPNSGGTNYAQKFQGRVTMTRDTSISTAYMELSRLRSDDTAVYYCARSPNPYYYDSSGYYYPGAFDIWGQGTMVTVSSASTKGPSVFPLAPSSKSTSGGTAALGCLVEDYFPEPVTVSWNSGALTSGVHTFPAVLQSSGLYSLSSVVTVPSSSLGTQTYICNVNHKPSNTKVDEKVEPKSCDKTHTCPPCPAPELLGGPSVFLFPPKPKDTLMISRTPEVTCVVVDVSHEDPEVKFNWYVDGVEVHNAKTKPREEQYNSTYRVVSVLTVLHQDWLNGKEYKCKVSNKALPAPIEKTISKAKGQPREPQVYTLPPCRDELTKNQVSLWCLVKGFYPSDIAVEWESNGQPENNYKTTPPVLDSDGSFFLYSKLTVDKSRWQQGNVFSCSVMHEALHNHYTQKSLSLSPGK

SEQ ID NO: 17 - protein, 212 aa, Artificial
  17938 - light chain (LC) <VEGF> with CL-CH1 domain exchange and Q38K substitution
DIQMTQSPSSLSASVGDRVTITCSASQDISNYLNWYQKKPGKAPKVLIYFTSSLHSGVPSRFSGSGSGTDFTLTISSLQPEDFATYYCQQYSTVPWTFGQGTKVEIKSSASTKGPSVFPLAPSSKSTSGGTAALGCLVKDYFPEPVTVSWNSGALTSGVHTFPAVLQSSGLYSLSSVVTVPSSSLGTQTYICNVNHKPSNTKVDKKVEPKSC

SEQ ID NO: 18 - protein, 457 aa, Artificial
  17936 - heavy chain (HC) <VEGF> with CL-CH1 domain exchange and Q39E substitution
EVQLVESGGGLVQPGGSLRLSCAASGYTFTNYGMNWVREAPGKGLEWVGWINTYTGEPTYAADFKRRFTFSLDTSKSTAYLQMNSLRAEDTAVYYCAKYPHYYGSSHWYFDVWGQGTLVTVSSASVAAPSVFIFPPSDEQLKSGTASVVCLLNNFYPREAKVQWKVDNALQSGNSQESVTEQDSKDSTYSLSSTLTLSKADYEKHKVYACEVTHQGLSSPVTKSFNRGECDKTHTCPPCPAPELLGGPSVFLFPPKPKDTLMISRTPEVTCVVVDVSHEDPEVKFNWYVDGVEVHNAKTKPREEQYNSTYRVVSVLTVLHQDWLNGKEYKCKVSNKALPAPIEKTISKAKGQPREPQVCTLPPSRDELTKNQVSLSCAVKGFYPSDIAVEWESNGQPENNYKTTPPVLDSDGSFFLVSKLTVDKSRWQQGNVFSCSVMHEALHNHYTQKSLSLSPGK

SEQ ID NO: 19 - protein, 215 aa, Artificial
  14098 - kappa light chain (LC) <Ang-2> with Q38K, E123K and Q124K substitutions
QPGLTQPPSVSVAPGQTARITCGGNNIGSKSVHWYQKKPGQAPVLVVYDDSDRPSGIPERFSGSNSGNTATLTISRVEAGDEADYYCQVWDSSSDHYVFGTGTKVTVLRTVAAPSVFIFPPSDKKLKSGTASVVCLLNNFYPREAKVQWKVDNALQSGNSQESVTEQDSKDSTYSLSSTLTLSKADYEKHKVYACEVTHQGLSSPVTKSFNRGEC

SEQ ID NO: 20 - protein, 459 aa, Artificial
  14097 - heavy chain (HC) <Ang-2> with Q39E, K147E and K213E substitutions
QVQLVESGAEVKKPGASVKVSCKASGYTFTGYYMHWVREAPGQGLEWMGWINPNSGGTNYAQKFQGRVTMTRDTSISTAYMELSRLRSDDTAVYYCARSPNPYYYDSSGYYYPGAFDIWGQGTMVTVSSASTKGPSVFPLAPSSKSTSGGTAALGCLVEDYFPEPVTVSWNSGALTSGVHTFPAVLQSSGLYSLSSVVTVPSSSLGTQTYICNVNHKPSNTKVDEKVEPKSCDKTHTCPPCPAPELLGGPSVFLFPPKPKDTLMISRTPEVTCVVVDVSHEDPEVKFNWYVDGVEVHNAKTKPREEQYNSTYRVVSVLTVLHQDWLNGKEYKCKVSNKALPAPIEKTISKAKGQPREPQVYTLPPCRDELTKNQVSLWCLVKGFYPSDIAVEWESNGQPENNYKTTPPVLDSDGSFFLYSKLTVDKSRWQQGNVFSCSVMHEALHNHYTQKSLSLSPGK

SEQ ID NO: 21 - protein, 457 aa, Artificial
  17937 - heavy chain (HC) <VEGF> with CL-CH1 domain exchange and with Q39E and Q124E substitutions
EVQLVESGGGLVQPGGSLRLSCAASGYTFTNYGMNWVREAPGKGLEWVGWINTYTGEPTYAADFKRRFTFSLDTSKSTAYLQMNSLRAEDTAVYYCAKYPHYYGSSHWYFDVWGQGTLVTVSSASVAAPSVFIFPPSDEELKSGTASVVCLLNNFYPREAKVQWKVDNALQSGNSQESVTEQDSKDSTYSLSSTLTLSKADYEKHKVYACEVTHQGLSSPVTKSFNRGECDKTHTCPPCPAPELLGGPSVFLFPPKPKDTLMISRTPEVTCVVVDVSHEDPEVKFNWYVDGVEVHNAKTKPREEQYNSTYRVVSVLTVLHQDWLNGKEYKCKVSNKALPAPIEKTISKAKGQPREPQVCTLPPSRDELTKNQVSLSCAVKGFYPSDIAVEWESNGQPENNYKTTPPVLDSDGSFFLVSKLTVDKSRWQQGNVFSCSVMHEALHNHYTQKSLSLSPGK

SEQ ID NO: 22 - protein, 215 aa, Artificial
  17962 - kappa light chain (LC) <Ang-2> with Q124E substitution
QPGLTQPPSVSVAPGQTARITCGGNNIGSKSVHWYQQKPGQAPVLVVYDDSDRPSGIPERFSGSNSGNTATLTISRVEAGDEADYYCQVWDSSSDHYVFGTGTKVTVLRTVAAPSVFIFPPSDEELKSGTASVVCLLNNFYPREAKVQWKVDNALQSGNSQESVTEQDSKDSTYSLSSTLTLSKADYEKHKVYACEVTHQGLSSPVTKSFNRGEC

SEQ ID NO: 23 - protein, 457 aa, Artificial
  17935 - heavy chain (HC) <VEGF> with CL-CH1 domain exchange and Q124E substitution
EVQLVESGGGLVQPGGSLRLSCAASGYTFTNYGMNWVRQAPGKGLEWVGWINTYTGEPTYAADFKRRFTFSLDTSKSTAYLQMNSLRAEDTAVYYCAKYPHYYGSSHWYFDVWGQGTLVTVSSASVAAPSVFIFPPSDEELKSGTASVVCLLNNFYPREAKVQWKVDNALQSGNSQESVTEQDSKDSTYSLSSTLTLSKADYEKHKVYACEVTHQGLSSPVTKSFNRGECDKTHTCPPCPAPELLGGPSVFLFPPKPKDTLMISRTPEVTCVVVDVSHEDPEVKFNWYVDGVEVHNAKTKPREEQYNSTYRVVSVLTVLHQDWLNGKEYKCKVSNKALPAPIEKTISKAKGQPREPQVCTLPPSRDELTKNQVSLSCAVKGFYPSDIAVEWESNGQPENNYKTTPPVLDSDGSFFLVSKLTVDKSRWQQGNVFSCSVMHEALHNHYTQKSLSLSPGK

SEQ ID NO: 24 - protein, 123 aa, Artificial [sequence omitted]

SEQ ID NO: 25 - protein, 107 aa, Artificial [sequence omitted]

SEQ ID NO: 26 - protein, 129 aa, Artificial
  variable heavy chain domain <Ang-2>
QVQLVESGAEVKKPGASVKVSCKASGYTFTGYYMHWVRQAPGQGLEWMGWINPNSGGTNYAQKFQGRVTMTRDTSISTAYMELSRLRSDDTAVYYCARSPNPYYYDSSGYYYPGAFDIWGQGTMVTVSS

SEQ ID NO: 27 - protein, 108 aa, Artificial
  variable light chain domain <Ang-2>
QPGLTQPPSVSVAPGQTARITCGGNNIGSKSVHWYQQKPGQAPVLVVYDDSDRPSGIPERFSGSNSGNTATLTISRVEAGDEADYYCQVWDSSSDHYVFGTGTKVTVL

SEQ ID NO: 28 - protein, 219 aa, Artificial
  6413 - IL17 LC E123 (Wt)/ Q124 (Wt)
DIVMTQSPLSLPVTPGEPASISCRSSQSLVHSNGDTYFHWYLQKPGQSPQLLIYKVSNRFSGVPDRFSGSGSGTDFTLKISRVEAEDVGVYYCSQTTHAPFTFGQGTKLEIKRTVAAPSVFIFPPSDEQLKSGTASVVCLLNNFYPREAKVQWKVDNALQSGNSQESVTEQDSKDSTYSLSSTLTLSKADYEKHKVYACEVTHQGLSSPVTKSFNRGEC

SEQ ID NO: 29 - protein, 448 aa, Artificial
  11738 - IL17 HC K147 (Wt)/ K213(Wt)
EVQLVESGGGLVQPGGSLRLSCAASGFSLDSYGVHWVRQATGKGLEWVSVIWSDGTTTYNSALKSRFTISRENAKNSLYLQMNSLRAGDTAVYYCARDTHYRLYYYAMDYWGQGTTVTVSSASTKGPSVFPLAPCSRSTSESTAALGCLVKDYFPEPVTVSWNSGALTSGVHTFPAVLQSSGLYSLSSVVTVPSSSLGTKTYTCNVDHKPSNTKVDKRVESKYGPPCPPCPAPEFEGGPSVFLFPPKPKDTLMISRTPEVTCVVVDVSQEDPEVQFNWYVDGVEVHNAKTKPREEQFNSTYRVVSVLTVLHQDWLNGKEYKCKVSNKGLPSSIEKTISKAKGQPREPQVCTLPPSQEEMTKNQVSLSCAVKGFYPSDIAVEWESNGQPENNYKTTPPVLDSDGSFFLVSRLTVDKSRWQEGNVFSCSVMHEALHNHYTQKSLSLSLGK

SEQ ID NO: 30 - protein, 216 aa, Artificial
  11755 - Tweak xLC K147(Wt)/ K213(Wt)
DIQMTQSPSSVSASVGDRVTITCQASQNIYSNLAWYQQKPGKAPKLLIYTASYLASGVPSRFSGSGSGTDYTLTISSLQPEDFATYYCQTAYYNSRPDTVAFGGGTKVEIKSSASTKGPSVFPLAPCSRSTSESTAALGCLVKDYFPEPVTVSWNSGALTSGVHTFPAVLQSSGLYSLSSVVTVPSSSLGTKTYTCNVDHKPSNTKVDKRVESKYG

SEQ ID NO: 31 - protein, 451 aa, Artificial
  11754 - Tweak xHC E123(Wt)/ Q124(Wt)
QVQLVQSGAEVKKPGSSVKVSCKASGFDFSTYYMSWVRQAPGQGLEWMGTVYVRQGTTYYASWLNGRVTITADESTSTAYMELSSLRSEDTAVYYCARGGYNYDDAFVIWGQGTLVTVSSASVAAPSVFIFPPSDEQLKSGTASVVCLLNNFYPREAKVQWKVDNALQSGNSQESVTEQDSKDSTYSLSSTLTLSKADYEKHKVYACEVTHQGLSSPVTKSFNRGECPPCPPCPAPEFEGGPSVFLFPPKPKDTLMISRTPEVTCVVVDVSQEDPEVQFNWYVDGVEVHNAKTKPREEQFNSTYRVVSVLTVLHQDWLNGKEYKCKVSNKGLPSSIEKTISKAKGQPREPQVYTLPPCQEEMTKNQVSLWCLVKGFYPSDIAVEWESNGQPENNYKTTPPVLDSDGSFFLYSRLTVDKSRWQEGNVFSCSVMHEALHNHYTQKSLSLSLGK

SEQ ID NO: 32 - protein, 219 aa, Artificial
  17843 - IL17 LC Q124K
DIVMTQSPLSLPVTPGEPASISCRSSQSLVHSNGDTYFHWYLQKPGQSPQLLIYKVSNRFSGVPDRFSGSGSGTDFTLKISRVEAEDVGVYYCSQTTHAPFTFGQGTKLEIKRTVAAPSVFIFPPSDEKLKSGTASVVCLLNNFYPREAKVQWKVDNALQSGNSQESVTEQDSKDSTYSLSSTLTLSKADYEKHKVYACEVTHQGLSSPVTKSFNRGEC

SEQ ID NO: 33 - protein, 448 aa, Artificial
  17844 - IL17 HC K147E
EVQLVESGGGLVQPGGSLRLSCAASGFSLDSYGVHWVRQATGKGLEWVSVIWSDGTTTYNSALKSRFTISRENAKNSLYLQMNSLRAGDTAVYYCARDTHYRLYYYAMDYWGQGTTVTVSSASTKGPSVFPLAPCSRSTSESTAALGCLVEDYFPEPVTVSWNSGALTSGVHTFPAVLQSSGLYSLSSVVTVPSSSLGTKTYTCNVDHKPSNTKVDKRVESKYGPPCPPCPAPEFEGGPSVFLFPPKPKDTLMISRTPEVTCVVVDVSQEDPEVQFNWYVDGVEVHNAKTKPREEQFNSTYRVVSVLTVLHQDWLNGKEYKCKVSNKGLPSSIEKTISKAKGQPREPQVCTLPPSQEEMTKNQVSLSCAVKGFYPSDIAVEWESNGQPENNYKTTPPVLDSDGSFFLVSRLTVDKSRWQEGNVFSCSVMHEALHNHYTQKSLSLSLGK

SEQ ID NO: 34 - protein, 448 aa, Artificial
  17845 - IL17 HC K213E
EVQLVESGGGLVQPGGSLRLSCAASGFSLDSYGVHWVRQATGKGLEWVSVIWSDGTTTYNSALKSRFTISRENAKNSLYLQMNSLRAGDTAVYYCARDTHYRLYYYAMDYWGQGTTVTVSSASTKGPSVFPLAPCSRSTSESTAALGCLVKDYFPEPVTVSWNSGALTSGVHTFPAVLQSSGLYSLSSVVTVPSSSLGTKTYTCNVDHKPSNTKVDERVESKYGPPCPPCPAPEFEGGPSVFLFPPKPKDTLMISRTPEVTCVVVDVSQEDPEVQFNWYVDGVEVHNAKTKPREEQFNSTYRVVSVLTVLHQDWLNGKEYKCKVSNKGLPSSIEKTISKAKGQPREPQVCTLPPSQEEMTKNQVSLSCAVKGFYPSDIAVEWESNGQPENNYKTTPPVLDSDGSFFLVSRLTVDKSRWQEGNVFSCSVMHEALHNHYTQKSLSLSLGK

SEQ ID NO: 35 - protein, 219 aa, Artificial
  17846 - IL17 LC E123K
DIVMTQSPLSLPVTPGEPASISCRSSQSLVHSNGDTYFHWYLQKPGQSPQLLIYKVSNRFSGVPDRFSGSGSGTDFTLKISRVEAEDVGVYYCSQTTHAPFTFGQGTKLEIKRTVAAPSVFIFPPSDKQLKSGTASVVCLLNNFYPREAKVQWKVDNALQSGNSQESVTEQDSKDSTYSLSSTLTLSKADYEKHKVYACEVTHQGLSSPVTKSFNRGEC

SEQ ID NO: 36 - protein, 219 aa, Artificial
  17847 - IL17 LC E123R / Q124K
DIVMTQSPLSLPVTPGEPASISCRSSQSLVHSNGDTYFHWYLQKPGQSPQLLIYKVSNRFSGVPDRFSGSGSGTDFTLKISRVEAEDVGVYYCSQTTHAPFTFGQGTKLEIKRTVAAPSVFIFPPSDKRLKSGTASVVCLLNNFYPREAKVQWKVDNALQSGNSQESVTEQDSKDSTYSLSSTLTLSKADYEKHKVYACEVTHQGLSSPVTKSFNRGEC

SEQ ID NO: 37 - protein, 448 aa, Artificial
  17848 - IL17 HC K147E / K213E
EVQLVESGGGLVQPGGSLRLSCAASGFSLDSYGVHWVRQATGKGLEWVSVIWSDGTTTYNSALKSRFTISRENAKNSLYLQMNSLRAGDTAVYYCARDTHYRLYYYAMDYWGQGTTVTVSSASTKGPSVFPLAPCSRSTSESTAALGCLVEDYFPEPVTVSWNSGALTSGVHTFPAVLQSSGLYSLSSVVTVPSSSLGTKTYTCNVDHKPSNTKVDERVESKYGPPCPPCPAPEFEGGPSVFLFPPKPKDTLMISRTPEVTCVVVDVSQEDPEVQFNWYVDGVEVHNAKTKPREEQFNSTYRVVSVLTVLHQDWLNGKEYKCKVSNKGLPSSIEKTISKAKGQPREPQVCTLPPSQEEMTKNQVSLSCAVKGFYPSDIAVEWESNGQPENNYKTTPPVLDSDGSFFLVSRLTVDKSRWQEGNVFSCSVMHEALHNHYTQKSLSLSLGK

SEQ ID NO: 38 - protein, 448 aa, Artificial
  17849 - IL17 HC K147E / K213D
EVQLVESGGGLVQPGGSLRLSCAASGFSLDSYGVHWVRQATGKGLEWVSVIWSDGTTTYNSALKSRFTISRENAKNSLYLQMNSLRAGDTAVYYCARDTHYRLYYYAMDYWGQGTTVTVSSASTKGPSVFPLAPCSRSTSESTAALGCLVEDYFPEPVTVSWNSGALTSGVHTFPAVLQSSGLYSLSSVVTVPSSSLGTKTYTCNVDHKPSNTKVDDRVESKYGPPCPPCPAPEFEGGPSVFLFPPKPKDTLMISRTPEVTCVVVDVSQEDPEVQFNWYVDGVEVHNAKTKPREEQFNSTYRVVSVLTVLHQDWLNGKEYKCKVSNKGLPSSIEKTISKAKGQPREPQVCTLPPSQEEMTKNQVSLSCAVKGFYPSDIAVEWESNGQPENNYKTTPPVLDSDGSFFLVSRLTVDKSRWQEGNVFSCSVMHEALHNHYTQKSLSLSLGK

SEQ ID NO: 39 - protein, 451 aa, Artificial
  17850 - Tweak xHC Q124E
QVQLVQSGAEVKKPGSSVKVSCKASGFDFSTYYMSWVRQAPGQGLEWMGTVYVRQGTTYYASWLNGRVTITADESTSTAYMELSSLRSEDTAVYYCARGGYNYDDAFVIWGQGTLVTVSSASVAAPSVFIFPPSDEELKSGTASVVCLLNNFYPREAKVQWKVDNALQSGNSQESVTEQDSKDSTYSLSSTLTLSKADYEKHKVYACEVTHQGLSSPVTKSFNRGECPPCPPCPAPEFEGGPSVFLFPPKPKDTLMISRTPEVTCVVVDVSQEDPEVQFNWYVDGVEVHNAKTKPREEQFNSTYRVVSVLTVLHQDWLNGKEYKCKVSNKGLPSSIEKTISKAKGQPREPQVYTLPPCQEEMTKNQVSLWCLVKGFYPSDIAVEWESNGQPENNYKTTPPVLDSDGSFFLYSRLTVDKSRWQEGNVFSCSVMHEALHNHYTQKSLSLSLGK